European Patent Specification EP 3 542 790 B1, published September 13, 2023. Title: Compositions comprising a delivery agent and preparation thereof. Applicant: Novo Nordisk A/S. The sequence listing filed with the application follows.

SEQUENCE LISTING (2 sequences)

SEQ ID NO: 1 - protein, 31 aa, Homo sapiens
HAEGTFTSDVSSYLEGQAAKEFIAWLVKGRG

SEQ ID NO: 2 - protein, 40 aa, Heloderma suspectum
HGEGTFITSDLSKQMEEEAVRLFIEWLKNGGPSSGAPPPS